European Patent Application EP 4 163 373 A1, published April 12, 2023. Title: SPLICE SHIFTING OLIGONUCLEOTIDES FOR USE IN THE TREATMENT OF DISEASES CHARACTERIZED BY ALTERED INCLUSION OF MICROEXONS. Applicant: Universidad Autónoma de Madrid Consejo Superior de Investigaciones Científicas University of Southern Denmark. The sequence listing filed with the application follows.

SEQUENCE LISTING (16 sequences)

SEQ ID NO: 1 - RNA, 23 nt, Artificial sequence
  Artificial sequence
uggaaacagugaagacugaccug

SEQ ID NO: 2 - RNA, 25 nt, Artificial sequence
  Artificial sequence
auuggaaacagugaagacugaccug

SEQ ID NO: 3 - RNA, 25 nt, Artificial sequence
  Artificial sequence
uggaaacagugaagacugaccugga

SEQ ID NO: 4 - RNA, 23 nt, Artificial sequence
  Artificial sequence
gaaacagugaagacugaccugga

SEQ ID NO: 5 - RNA, 23 nt, Artificial sequence
  Artificial sequence
ggaaacagugaagacugaccugg

SEQ ID NO: 6 - RNA, 21 nt, Artificial sequence
  Artificial sequence
aaacagugaagacugaccugg

SEQ ID NO: 7 - RNA, 19 nt, Artificial sequence
  Artificial sequence
acagugaagacugaccugg

SEQ ID NO: 8 - RNA, 18 nt, Artificial sequence
  Artificial sequence
cagugaagacugaccugg

SEQ ID NO: 9 - RNA, 18 nt, Artificial sequence
  Artificial sequence
ugccacugauuaucaugc

SEQ ID NO: 10 - RNA, 18 nt, Artificial sequence
  Artificial sequence
aaagaaacaaggaaacag

SEQ ID NO: 11 - RNA, 18 nt, Artificial sequence
  Artificial sequence
uccaagaauccaucuucc

SEQ ID NO: 12 - RNA, 18 nt, Artificial sequence
  Artificial sequence
ugauccccacggccauca

SEQ ID NO: 13 - RNA, 20 nt, Artificial sequence
  Artificial sequence
cucaauaugcuacugccaug

SEQ ID NO: 14 - DNA, 21 bp, Artificial sequence
  Artificial sequence
ggacgtttgacatgcactcac

SEQ ID NO: 15 - DNA, 18 bp, Artificial sequence
  Artificial sequence
gaggttgatccccacggc

SEQ ID NO: 16 - DNA, 20 bp, Artificial sequence
  Artificial sequence
ccaaagcgacgaaaactagc